European Patent Application EP 4 382 619 A2, published June 12, 2024. Title: COMPOSITIONS, METHODS AND KITS TO DETECT RHINOVIRUS NUCLEIC ACIDS. Applicant: Gen-Probe Incorporated. Application EP 23156456.8, filed March 23, 2018. The sequence listing filed with the application follows.

SEQUENCE LISTING (178 sequences)

SEQ ID NO: 1 - DNA, 23 bp, synthetic construct
  misc_feature 1..23: note = Synthetic Oligonucleotide
  source 1..23: mol_type = other DNA
caggacgcctcggrgtayctsag

SEQ ID NO: 2 - DNA, 17 bp, synthetic construct
  misc_feature 1..17: note = Synthetic Oligonucleotide
  source 1..17: mol_type = other DNA
ggagccacvgtgggrtt

SEQ ID NO: 3 - DNA, 17 bp, synthetic construct
  misc_feature 1..17: note = Synthetic Oligonucleotide
  source 1..17: mol_type = other DNA
aaycccacbgtggctcc

SEQ ID NO: 4 - DNA, 24 bp, synthetic construct
  misc_feature 1..24: note = Synthetic Oligonucleotide
  source 1..24: mol_type = other DNA
ccgggtctggtgcagtttgcccgc

SEQ ID NO: 5 - DNA, 17 bp, synthetic construct
  misc_feature 1..17: note = Synthetic Oligonucleotide
  source 1..17: mol_type = other DNA
cacatcgccggacagga

SEQ ID NO: 6 - DNA, 21 bp, synthetic construct
  misc_feature 1..21: note = Synthetic Oligonucleotide
  source 1..21: mol_type = other DNA
catactgaagtaggtgtctgt

SEQ ID NO: 7 - DNA, 21 bp, synthetic construct
  misc_feature 1..21: note = Synthetic Oligonucleotide
  source 1..21: mol_type = other DNA
acagacacctacttcagtatg

SEQ ID NO: 8 - DNA, 17 bp, synthetic construct
  misc_feature 1..17: note = Synthetic Oligonucleotide
  source 1..17: mol_type = other DNA
cggtggtcacatcgtgg

SEQ ID NO: 9 - DNA, 17 bp, synthetic construct
  misc_feature 1..17: note = Synthetic Oligonucleotide
  source 1..17: mol_type = other DNA
ccacgatgtgaccaccg

SEQ ID NO: 10 - DNA, 23 bp, synthetic construct
  misc_feature 1..23: note = Synthetic Oligonucleotide
  source 1..23: mol_type = other DNA
agtacctcagtccgggtctggtg

SEQ ID NO: 11 - DNA, 18 bp, synthetic construct
  misc_feature 1..18: note = Synthetic Oligonucleotide
  source 1..18: mol_type = other DNA
atggctaccccttcgatg

SEQ ID NO: 12 - DNA, 17 bp, synthetic construct
  misc_feature 1..17: note = Synthetic Oligonucleotide
  source 1..17: mol_type = other DNA
accccmtcgatgatgcc

SEQ ID NO: 13 - DNA, 17 bp, synthetic construct
  misc_feature 1..17: note = Synthetic Oligonucleotide
  source 1..17: mol_type = other DNA
gcgggcgaattgcacca

SEQ ID NO: 14 - DNA, 17 bp, synthetic construct
  misc_feature 1..17: note = Synthetic Oligonucleotide
  source 1..17: mol_type = other DNA
tggtgcaattcgcccgc

SEQ ID NO: 15 - DNA, 17 bp, synthetic construct
  misc_feature 1..17: note = Synthetic Oligonucleotide
  source 1..17: mol_type = other DNA
gcgggcaaaytgcacca

SEQ ID NO: 16 - DNA, 17 bp, synthetic construct
  misc_feature 1..17: note = Synthetic Oligonucleotide
  source 1..17: mol_type = other DNA
tggtgcartttgcccgc

SEQ ID NO: 17 - DNA, 24 bp, synthetic construct
  misc_feature 1..24: note = Synthetic Oligonucleotide
  source 1..24: mol_type = other DNA
gactcaggtactccgaagcatcct

SEQ ID NO: 18 - DNA, 24 bp, synthetic construct
  misc_feature 1..24: note = Synthetic Oligonucleotide
  source 1..24: mol_type = other DNA
aggatgcttcggagtacctgagtc

SEQ ID NO: 19 - DNA, 22 bp, synthetic construct
  misc_feature 1..22: note = Synthetic Oligonucleotide
  source 1..22: mol_type = other DNA
ctcaggtactccgaggcgtcct

SEQ ID NO: 20 - DNA, 22 bp, synthetic construct
  misc_feature 1..22: note = Synthetic Oligonucleotide
  source 1..22: mol_type = other DNA
aggacgcctcggagtacctgag

SEQ ID NO: 21 - DNA, 22 bp, synthetic construct
  misc_feature 1..22: note = Synthetic Oligonucleotide
  source 1..22: mol_type = other DNA
ctcaggtactccgaagcatcct

SEQ ID NO: 22 - DNA, 22 bp, synthetic construct
  misc_feature 1..22: note = Synthetic Oligonucleotide
  source 1..22: mol_type = other DNA
aggatgcttcggagtacctgag

SEQ ID NO: 23 - DNA, 20 bp, synthetic construct
  misc_feature 1..20: note = Synthetic Oligonucleotide
  source 1..20: mol_type = other DNA
caggtactccgaggcgtcct

SEQ ID NO: 24 - DNA, 20 bp, synthetic construct
  misc_feature 1..20: note = Synthetic Oligonucleotide
  source 1..20: mol_type = other DNA
aggacgcctcggagtacctg

SEQ ID NO: 25 - DNA, 17 bp, synthetic construct
  misc_feature 1..17: note = Synthetic Oligonucleotide
  source 1..17: mol_type = other DNA
accccatcgatgatgcc

SEQ ID NO: 26 - DNA, 17 bp, synthetic construct
  misc_feature 1..17: note = Synthetic Oligonucleotide
  source 1..17: mol_type = other DNA
accccctcgatgatgcc

SEQ ID NO: 27 - DNA, 17 bp, synthetic construct
  misc_feature 1..17: note = Synthetic Oligonucleotide
  source 1..17: mol_type = other DNA
gcgggcaaactgcacca

SEQ ID NO: 28 - DNA, 17 bp, synthetic construct
  misc_feature 1..17: note = Synthetic Oligonucleotide
  source 1..17: mol_type = other DNA
gcgggcaaattgcacca

SEQ ID NO: 29 - DNA, 22 bp, synthetic construct
  misc_feature 1..22: note = Synthetic Oligonucleotide
  source 1..22: mol_type = other DNA
ctcaggtattccgaggcatcct

SEQ ID NO: 30 - DNA, 22 bp, synthetic construct
  misc_feature 1..22: note = Synthetic Oligonucleotide
  source 1..22: mol_type = other DNA
aggatgcctcggaatacctgag

SEQ ID NO: 31 - DNA, 17 bp, synthetic construct
  misc_feature 1..17: note = Synthetic Oligonucleotide
  source 1..17: mol_type = other DNA
accccatcgatgctgcc

SEQ ID NO: 32 - DNA, 17 bp, synthetic construct
  misc_feature 1..17: note = Synthetic Oligonucleotide
  source 1..17: mol_type = other DNA
accccatcgatgatgcc

SEQ ID NO: 33 - DNA, 18 bp, synthetic construct
  misc_feature 1..18: note = Synthetic Oligonucleotide
  source 1..18: mol_type = other DNA
tgggcgtacatgcacatc

SEQ ID NO: 34 - DNA, 19 bp, synthetic construct
  misc_feature 1..19: note = Synthetic Oligonucleotide
  source 1..19: mol_type = other DNA
gtggtcttacatgcacatc

SEQ ID NO: 35 - DNA, 19 bp, synthetic construct
  misc_feature 1..19: note = Synthetic Oligonucleotide
  source 1..19: mol_type = other DNA
gtgggcatacatgcacatc

SEQ ID NO: 36 - DNA, 22 bp, synthetic construct
  misc_feature 1..22: note = Synthetic Oligonucleotide
  source 1..22: mol_type = other DNA
aggatgcttcggagtacctgag

SEQ ID NO: 37 - DNA, 20 bp, synthetic construct
  misc_feature 1..20: note = Synthetic Oligonucleotide
  source 1..20: mol_type = other DNA
aggacgcctcggagtacctg

SEQ ID NO: 38 - DNA, 20 bp, synthetic construct
  misc_feature 1..20: note = Synthetic Oligonucleotide
  source 1..20: mol_type = other DNA
artggkcdtacatgcacatc

SEQ ID NO: 39 - DNA, 20 bp, synthetic construct
  misc_feature 1..20: note = Synthetic Oligonucleotide
  source 1..20: mol_type = other DNA
caggacgcctcggagtacct

SEQ ID NO: 40 - DNA, 22 bp, synthetic construct
  misc_feature 1..22: note = Synthetic Oligonucleotide
  source 1..22: mol_type = other DNA
aggatgcttcggagtacctgag

SEQ ID NO: 41 - DNA, 17 bp, synthetic construct
  misc_feature 1..17: note = Synthetic Oligonucleotide
  source 1..17: mol_type = other DNA
cacgatgtgaccacaga

SEQ ID NO: 42 - DNA, 17 bp, synthetic construct
  misc_feature 1..17: note = Synthetic Oligonucleotide
  source 1..17: mol_type = other DNA
caygatgtgaccacaga

SEQ ID NO: 43 - DNA, 17 bp, synthetic construct
  misc_feature 1..17: note = Synthetic Oligonucleotide
  source 1..17: mol_type = other DNA
cacgaygtgaccacaga

SEQ ID NO: 44 - DNA, 17 bp, synthetic construct
  misc_feature 1..17: note = Synthetic Oligonucleotide
  source 1..17: mol_type = other DNA
cacgatgtgaccacsga

SEQ ID NO: 45 - DNA, 17 bp, synthetic construct
  misc_feature 1..17: note = Synthetic Oligonucleotide
  source 1..17: mol_type = other DNA
cacgatgtgaccacvga

SEQ ID NO: 46 - DNA, 17 bp, synthetic construct
  misc_feature 1..17: note = Synthetic Oligonucleotide
  source 1..17: mol_type = other DNA
caygaygtgaccacvga

SEQ ID NO: 47 - DNA, 2832 bp, Human adenovirus type 9
  source 1..2832: mol_type = unassigned DNA
atggccaccccctcgatgatgccgcagtgggcgtacatgcacatcgccgggcaggacgcctcggagtacctgagcccgggtctggtgcagtttgcccgcgccaccgacacgtacttcagcctgggcaacaagtttaggaaccccacggtggccccgacccacgatgtgaccacggaccggtcccagcgtctgacgctgcgcttcgtgcccgtggatcgcgaggacaccacgtactcgtacaaggcgcgcttcactctggccgtgggcgacaaccgggtgctagacatggccagcacttactttgacatccgcggcgtcctggaccgcggtcccagcttcaaaccctactcgggcacagcttacaacagtctggcccccaagggtgcccccaactccagccagtggcttgcaaaagacaccaatgctggcgatcaagcattaaaaacccacacacatggcgtagctgctatggggggaacagatatcacagcaaagggtttgcaaattggtgttgacacgactgaaaacaagaatgagcctatttatgcaaatgaaatataccagccagaacctcaggtaggagaggaaaacttgcaagatgttgaaaacttttatggaggcagagctcttaaaaaagaaaccaaaatgaaaccttgctatggctcgtttgccagacccacaaatgaaaaaggcggtcaagccaaatttttaactgacggcgatggtcagctaactaaaaatcatgatatcacaatgaatttctttgacactcctggaggaacagttggtcaggatactgaacttgaagcagacattgttatgtatgctgagaatgtgcatctggaaactccagacacgcatgtggtgtacaaaccaggaacttctgatgagagttcagaagcaaatttggttcagcagtccatgccaaacaggcccaactacatcggcttcagggacaactttgtgggtctcatgtactataacagcactggcaacatgggtgtgctggctggtcaagcatctcagttgaatgctgtggtcgacttgcaagacagaaacacagagctgtcttaccagctcttgctagattctctgggtgacagaaccagatactttagcatgtggaactctgcagtggacagttatgatcctgatgtcaggattattgaaaatcacggtgtggaagatgaacttccaaactattgcttcccattggatggagctggcactaatgctacctaccaaggtgtaaaagttaaaaatggccaagatggagatgtaaacgcagattgggaaaaagatccaaatcttgcttcacgaaaccaaatatgcaagggtaacatcttcgccatggagatcaacctccaggccaacctgtggaagagttttctgtactcgaatgtggccctgtacctgcccgactcatacaagtacacgccggccaacgtcacgctgcccgccaataccaacacctacgagtacatgaacggccgcgtggtagccccctcgctggtggacgcctacatcaacatcggcgcccggtggtcgctggaccccatggacaacgtcaacccattcaaccaccaccgcaacgcgggcctgcgttaccgctccatgcttctgggcaacggccgctacgtgcccttccacatccaagtgccccaaaagttctttgccatcaagaacctgctcctgctccccggctcctacacctacgagtggaacttccgcaaggatgtcaacatgatcctgcagagttccctcggaaacgacctgcgcgtcgacggcgcctccgtccgcttcgacagcgtcaacctctacgccacattcttccccatggcgcacaacaccgcctccaccctggaagccatgctgcgcaacgacaccaacgaccagtccttcaacgactacctctcggccgccaacatgctctaccccatcccggccaaggccaccaacgtgcccatctccatcccctcgcgcaactgggccgccttccgcggctggagtttcacccggctcaagaccaaagaaactccctccctcggctcgggtttcgatccctactttgtatactcgggttccatcccctacctcgacgggaccttctacctcaaccacaccttcaagaaggtctccatcatgttcgactcctcggtcagctggcccggcaacgaccggctgctcacgccgaacgagttcgagatcaagcgcagtgtcgacggggagggctacaatgtggcccaatgcaacatgaccaaggactggttcctcgtccagatgctctcccactacaacatcggctaccagggcttccacgtgcccgagggctacaaggaccgcatgtactccttcttccgcaacttccagcccatgagcaggcaggtggtcgatgagatcaactacaaggactacaaggccgtcaccctgcccttccagcacaacaactcgggcttcaccggctaccttgcacccaccatgcgtcaggggcagccctaccccgccaacttcccctatcctctcatcggccagacagccgtgccctctgtcacccagaaaaagttcctctgcgacagggtcatgtggcgcatccccttctccagcaacttcatgtccatgggcgccctcaccgacctgggtcagaacatgctctatgccaactcggcccacgcgctcgacatgaccttcgaggtggaccccatggatgagcccaccctcctctatcttctcttcgaagttttcgacgtggtcagagtgcaccagccgcaccgcggcgtcatcgaggccgtctacctgcgcacgcccttctccgccggcaacgccaccacctaa

SEQ ID NO: 48 - DNA, 17 bp, synthetic construct
  misc_feature 1..17: note = Synthetic Oligonucleotide
  source 1..17: mol_type = other DNA
agcctgcgtggcggcca

SEQ ID NO: 49 - DNA, 20 bp, synthetic construct
  misc_feature 1..20: note = Synthetic Oligonucleotide
  source 1..20: mol_type = other DNA
  modified_base 17: mod_base = OTHER; note = uracil
  modified_base 5: mod_base = OTHER; note = uracil
agcctgcgtggtgccctgcc

SEQ ID NO: 50 - DNA, 22 bp, synthetic construct
  misc_feature 1..22: note = Synthetic Oligonucleotide
  source 1..22: mol_type = other DNA
  modified_base 8: mod_base = OTHER; note = uracil
cactagtttggtcgatgaggct

SEQ ID NO: 51 - DNA, 27 bp, synthetic construct
  misc_feature 1..27: note = Synthetic Oligonucleotide
  source 1..27: mol_type = other DNA
  modified_base 18: mod_base = OTHER; note = uracil
ccatctgtagattagggtaatgaggct

SEQ ID NO: 52 - DNA, 26 bp, synthetic construct
  misc_feature 1..26: note = Synthetic Oligonucleotide
  source 1..26: mol_type = other DNA
cccaactttgcaagtgttgttctcgg

SEQ ID NO: 53 - DNA, 27 bp, synthetic construct
  misc_feature 1..27: note = Synthetic Oligonucleotide
  source 1..27: mol_type = other DNA
ccccaattttgctagtgttgttcttgg

SEQ ID NO: 54 - DNA, 17 bp, synthetic construct
  misc_feature 1..17: note = Synthetic Oligonucleotide
  source 1..17: mol_type = other DNA
  modified_base 3: mod_base = OTHER; note = uracil
cctgcgtggctgcctgc

SEQ ID NO: 55 - DNA, 28 bp, synthetic construct
  misc_feature 1..28: note = Synthetic Oligonucleotide
  source 1..28: mol_type = other DNA
cgtcgaccgaagtcctgcaaaaggtcac

SEQ ID NO: 56 - DNA, 28 bp, synthetic construct
  misc_feature 1..28: note = Synthetic Oligonucleotide
  source 1..28: mol_type = other DNA
ctgctgctgaaaatagttctgtgtttgg

SEQ ID NO: 57 - DNA, 23 bp, synthetic construct
  misc_feature 1..23: note = Synthetic Oligonucleotide
  source 1..23: mol_type = other DNA
gaaacacggacacccaaagtagt

SEQ ID NO: 58 - DNA, 21 bp, synthetic construct
  misc_feature 1..21: note = Synthetic Oligonucleotide
  source 1..21: mol_type = other DNA
ggcctctgctaaagcaacacc

SEQ ID NO: 59 - DNA, 21 bp, synthetic construct
  misc_feature 1..21: note = Synthetic Oligonucleotide
  source 1..21: mol_type = other DNA
gtagatcggggcaatggggct

SEQ ID NO: 60 - DNA, 21 bp, synthetic construct
  misc_feature 1..21: note = Synthetic Oligonucleotide
  source 1..21: mol_type = other DNA
gtagatcggggtaatggggct

SEQ ID NO: 61 - DNA, 18 bp, synthetic construct
  misc_feature 1..18: note = Synthetic Oligonucleotide
  source 1..18: mol_type = other DNA
gtggcgcgggcgaactgc

SEQ ID NO: 62 - DNA, 18 bp, synthetic construct
  misc_feature 1..18: note = Synthetic Oligonucleotide
  source 1..18: mol_type = other DNA
gttgcacgggcgaactgc

SEQ ID NO: 63 - DNA, 23 bp, synthetic construct
  misc_feature 1..23: note = Synthetic Oligonucleotide
  source 1..23: mol_type = other DNA
tacatgcacatcgccgggcagga

SEQ ID NO: 64 - DNA, 23 bp, synthetic construct
  misc_feature 1..23: note = Synthetic Oligonucleotide
  source 1..23: mol_type = other DNA
tacatgcacatctcgggccagga

SEQ ID NO: 65 - DNA, 19 bp, synthetic construct
  misc_feature 1..19: note = Synthetic Oligonucleotide
  source 1..19: mol_type = other DNA
tagacctggcagatgaggc

SEQ ID NO: 66 - DNA, 19 bp, synthetic construct
  misc_feature 1..19: note = Synthetic Oligonucleotide
  source 1..19: mol_type = other DNA
tgccgcagaacgttgcgaa

SEQ ID NO: 67 - DNA, 33 bp, synthetic construct
  misc_feature 1..33: note = Synthetic Oligonucleotide
  source 1..33: mol_type = other DNA
tgcctcaggcttaggcataataggtatgtatcg

SEQ ID NO: 68 - DNA, 27 bp, synthetic construct
  misc_feature 1..27: note = Synthetic Oligonucleotide
  source 1..27: mol_type = other DNA
tgctgcagaaaatagctctgtgtttgg

SEQ ID NO: 69 - DNA, 33 bp, synthetic construct
  misc_feature 1..33: note = Synthetic Oligonucleotide
  source 1..33: mol_type = other DNA
tgcttcaggtctaggtataatcggaatgtacag

SEQ ID NO: 70 - DNA, 33 bp, synthetic construct
  misc_feature 1..33: note = Synthetic Oligonucleotide
  source 1..33: mol_type = other DNA
tgcttcaggtttaggcataatcggaatgtacag

SEQ ID NO: 71 - DNA, 20 bp, synthetic construct
  misc_feature 1..20: note = Synthetic Oligonucleotide
  source 1..20: mol_type = other DNA
tggccactccgtcgatgatg

SEQ ID NO: 72 - DNA, 20 bp, synthetic construct
  misc_feature 1..20: note = Synthetic Oligonucleotide
  source 1..20: mol_type = other DNA
tggctaccccatcgatgatg

SEQ ID NO: 73 - DNA, 20 bp, synthetic construct
  misc_feature 1..20: note = Synthetic Oligonucleotide
  source 1..20: mol_type = other DNA
tggctaccccatcgatgctg

SEQ ID NO: 74 - DNA, 19 bp, synthetic construct
  misc_feature 1..19: note = Synthetic Oligonucleotide
  source 1..19: mol_type = other DNA
  modified_base 11: mod_base = OTHER; note = uracil
tggctacccctcgatgatg

SEQ ID NO: 75 - DNA, 20 bp, synthetic construct
  misc_feature 1..20: note = Synthetic Oligonucleotide
  source 1..20: mol_type = other DNA
  modified_base 6: mod_base = OTHER; note = uracil
ctagtttggtcgatgaggct

SEQ ID NO: 76 - DNA, 425 bp, Human rhinovirus
  source 1..425: mol_type = unassigned DNA
ggtgtgtgaatagactctaacagggttgaagctgtagcactcgttatccgcacaactactacgcgaatgttagtaacaccctctaggtatagtgggatttcgctccgcagaaaccccatctgtagattagggtaatgaggctacacagaccccactggcgacagtggtgtagcctgcgtggtgccctacctggggtttctcaccccaggattccactttactgacagggtgtgaaggcgctagtgtgctagttgtgagtcctccggtccctgaatgtggctaatcctaaccccgtggccatttcatgtaatccaacatgcaggtggtcgtaacgagcaatcacgggatggaaccaactactttgggtaaccgtgtttcctgttttactttaatgtgtgtcttatggttacaattatagagtaacc

SEQ ID NO: 77 - DNA, 29 bp, synthetic construct
  misc_feature 1..29: note = Synthetic Oligonucleotide
  source 1..29: mol_type = other DNA
ccatctgtagrtyrgggyaatgrggctac

SEQ ID NO: 78 - DNA, 23 bp, synthetic construct
  misc_feature 1..23: note = Synthetic Oligonucleotide
  source 1..23: mol_type = other DNA
  modified_base 12: mod_base = OTHER; note = uracil
gtagattagggtaatgaggctac

SEQ ID NO: 79 - DNA, 21 bp, synthetic construct
  misc_feature 1..21: note = Synthetic Oligonucleotide
  source 1..21: mol_type = other DNA
  modified_base 12: mod_base = OTHER; note = uracil
gtagattagggtaatgaggct

SEQ ID NO: 80 - DNA, 21 bp, synthetic construct
  misc_feature 1..21: note = Synthetic Oligonucleotide
  source 1..21: mol_type = other DNA
  modified_base 12: mod_base = OTHER; note = uracil
gtagatcrgggtaatggggct

SEQ ID NO: 81 - DNA, 21 bp, synthetic construct
  misc_feature 1..21: note = Synthetic Oligonucleotide
  source 1..21: mol_type = other DNA
gtagatcrgggyaatggggct

SEQ ID NO: 82 - DNA, 21 bp, synthetic construct
  misc_feature 1..21: note = Synthetic Oligonucleotide
  source 1..21: mol_type = other DNA
  modified_base 12: mod_base = OTHER; note = uracil
gtagatcrgggtaatgrggct

SEQ ID NO: 83 - DNA, 23 bp, synthetic construct
  misc_feature 1..23: note = Synthetic Oligonucleotide
  source 1..23: mol_type = other DNA
gtagatcggggtaatggggctac

SEQ ID NO: 84 - DNA, 23 bp, synthetic construct
  misc_feature 1..23: note = Synthetic Oligonucleotide
  source 1..23: mol_type = other DNA
gtagatcggggcaatggggctac

SEQ ID NO: 85 - DNA, 19 bp, synthetic construct
  misc_feature 1..19: note = Synthetic Oligonucleotide
  source 1..19: mol_type = other DNA
gtagatcrgggyaatgrgg

SEQ ID NO: 86 - DNA, 23 bp, synthetic construct
  misc_feature 1..23: note = Synthetic Oligonucleotide
  source 1..23: mol_type = other DNA
gtagatcrgggyaatgrggctac

SEQ ID NO: 87 - DNA, 20 bp, synthetic construct
  misc_feature 1..20: note = Synthetic Oligonucleotide
  source 1..20: mol_type = other DNA
agcctgcgtggyksccwrcc

SEQ ID NO: 88 - DNA, 20 bp, synthetic construct
  misc_feature 1..20: note = Synthetic Oligonucleotide
  source 1..20: mol_type = other DNA
agccygcgtggtgcccygcc

SEQ ID NO: 89 - DNA, 17 bp, synthetic construct
  misc_feature 1..17: note = Synthetic Oligonucleotide
  source 1..17: mol_type = other DNA
  modified_base 2: mod_base = OTHER; note = uracil
ctgcgtggtgcccygcc

SEQ ID NO: 90 - DNA, 17 bp, synthetic construct
  misc_feature 1..17: note = Synthetic Oligonucleotide
  source 1..17: mol_type = other DNA
  modified_base 14: mod_base = OTHER; note = uracil
cygcgtggtgccctgcc

SEQ ID NO: 91 - DNA, 14 bp, synthetic construct
  misc_feature 1..14: note = Synthetic Oligonucleotide
  source 1..14: mol_type = other DNA
agccygcgtggtgc

SEQ ID NO: 92 - DNA, 17 bp, synthetic construct
  misc_feature 1..17: note = Synthetic Oligonucleotide
  source 1..17: mol_type = other DNA
agcctgcgtggcggcca

SEQ ID NO: 93 - DNA, 16 bp, synthetic construct
  misc_feature 1..16: note = Synthetic Oligonucleotide
  source 1..16: mol_type = other DNA
agccygcgtggtgccc

SEQ ID NO: 94 - DNA, 17 bp, synthetic construct
  misc_feature 1..17: note = Synthetic Oligonucleotide
  source 1..17: mol_type = other DNA
  modified_base 3: mod_base = OTHER; note = uracil
cctgcgtggctgcctgc

SEQ ID NO: 95 - DNA, 27 bp, synthetic construct
  misc_feature 1..27: note = Synthetic Oligonucleotide
  source 1..27: mol_type = other DNA
grttagccrcattcaggggccggagga

SEQ ID NO: 96 - DNA, 35 bp, synthetic construct
  misc_feature 1..35: note = Synthetic Oligonucleotide
  source 1..35: mol_type = other DNA
gaaacacggacacccaaagtagtyggtyccrtccc

SEQ ID NO: 97 - DNA, 19 bp, synthetic construct
  misc_feature 1..19: note = Synthetic Oligonucleotide
  source 1..19: mol_type = other DNA
aagtagttggtcccatccc

SEQ ID NO: 98 - DNA, 19 bp, synthetic construct
  misc_feature 1..19: note = Synthetic Oligonucleotide
  source 1..19: mol_type = other DNA
aagtagttggttccatccc

SEQ ID NO: 99 - DNA, 19 bp, synthetic construct
  misc_feature 1..19: note = Synthetic Oligonucleotide
  source 1..19: mol_type = other DNA
aagtagtcggtcccatccc

SEQ ID NO: 100 - DNA, 19 bp, synthetic construct
  misc_feature 1..19: note = Synthetic Oligonucleotide
  source 1..19: mol_type = other DNA
aagtagttggtcccgtccc

SEQ ID NO: 101 - DNA, 549 bp, Human rhinovirus
  source 1..549: mol_type = unassigned DNA
ttcctaatgtacccaccctaaaacttcctacccaagtaacgttagaagtttcatcaacaagtacaataggaagcatcacatccagtggtgttttgtacaagcacttctgtttccccggagcgaggtataggctgtacccactgccgaaagcctttaaccgttatccgccaaccaactacgtaaaagctagtatcatcatgttttaaaataggcgttcgatcaggtggatcccccctccactagtttggtcgatgaggctaggaactccccacgggtgaccgtgtcctagcctgcgtggcggccaacccagcttctgctgggacgcctttttatggacatggtgtgaagactcgcatgtgcttggttgtgactcctccggcccctgaatgcggctaaccttaaccccggagccctgtgttgcaatccagtaacattagggtcgtaatgagcaatttcgggacgggaccgactactttgggtgtccgtgtttctcatttttcttattattgtcttatggtcacagcatatatataacgtatatactgtgat

SEQ ID NO: 102 - DNA, 22 bp, synthetic construct
  misc_feature 1..22: note = Synthetic Oligonucleotide
  source 1..22: mol_type = other DNA
cactagtttggycgatgaggct

SEQ ID NO: 103 - DNA, 19 bp, synthetic construct
  misc_feature 1..19: note = Synthetic Oligonucleotide
  source 1..19: mol_type = other DNA
ctagtytggtcgatgaggc

SEQ ID NO: 104 - DNA, 18 bp, synthetic construct
  misc_feature 1..18: note = Synthetic Oligonucleotide
  source 1..18: mol_type = other DNA
ctagtytggtcgatgagg

SEQ ID NO: 105 - DNA, 16 bp, synthetic construct
  misc_feature 1..16: note = Synthetic Oligonucleotide
  source 1..16: mol_type = other DNA
gtytggtcgatgaggc

SEQ ID NO: 106 - DNA, 19 bp, synthetic construct
  misc_feature 1..19: note = Synthetic Oligonucleotide
  source 1..19: mol_type = other DNA
tagtytggtcgatgaggct

SEQ ID NO: 107 - DNA, 19 bp, synthetic construct
  misc_feature 1..19: note = Synthetic Oligonucleotide
  source 1..19: mol_type = other DNA
  modified_base 5: mod_base = OTHER; note = uracil
tagtttggtcgatgaggct

SEQ ID NO: 108 - DNA, 18 bp, synthetic construct
  misc_feature 1..18: note = Synthetic Oligonucleotide
  source 1..18: mol_type = other DNA
rcattcaggggccggagg

SEQ ID NO: 109 - DNA, 20 bp, synthetic construct
  misc_feature 1..20: note = Synthetic Oligonucleotide
  source 1..20: mol_type = other DNA
agcctgcgtggcggccarcc

SEQ ID NO: 110 - DNA, 17 bp, synthetic construct
  misc_feature 1..17: note = Synthetic Oligonucleotide
  source 1..17: mol_type = other DNA
  modified_base 3: mod_base = OTHER; note = uracil
cctgcgtggctgcctrc

SEQ ID NO: 111 - DNA, 17 bp, synthetic construct
  misc_feature 1..17: note = Synthetic Oligonucleotide
  source 1..17: mol_type = other DNA
ctgcgtggtgccctacc

SEQ ID NO: 112 - DNA, 17 bp, synthetic construct
  misc_feature 1..17: note = Synthetic Oligonucleotide
  source 1..17: mol_type = other DNA
ccygcgtggctgcctac

SEQ ID NO: 113 - DNA, 14 bp, synthetic construct
  misc_feature 1..14: note = Synthetic Oligonucleotide
  source 1..14: mol_type = other DNA
agccygcgtggctg

SEQ ID NO: 114 - DNA, 16 bp, synthetic construct
  misc_feature 1..16: note = Synthetic Oligonucleotide
  source 1..16: mol_type = other DNA
agccygcgtggctgcc

SEQ ID NO: 115 - DNA, 27 bp, synthetic construct
  misc_feature 1..27: note = Synthetic Oligonucleotide
  source 1..27: mol_type = other DNA
grttagccrcattcrggrgccggagga

SEQ ID NO: 116 - DNA, 18 bp, synthetic construct
  misc_feature 1..18: note = Synthetic Oligonucleotide
  source 1..18: mol_type = other DNA
gcattcaggggccggagg

SEQ ID NO: 117 - DNA, 26 bp, synthetic construct
  misc_feature 1..26: note = Synthetic Oligonucleotide
  source 1..26: mol_type = other DNA
gaaacacggacacccaaagtagtygg

SEQ ID NO: 118 - DNA, 29 bp, synthetic construct
  misc_feature 1..29: note = Synthetic Oligonucleotide
  source 1..29: mol_type = other DNA
gaaacacggacacccaaagtagtyggtcc

SEQ ID NO: 119 - DNA, 19 bp, synthetic construct
  misc_feature 1..19: note = Synthetic Oligonucleotide
  source 1..19: mol_type = other DNA
aagtagtcggtcccgtccc

SEQ ID NO: 120 - DNA, 576 bp, Human rhinovirus
  source 1..576: mol_type = unassigned DNA
tggatttcccacaggagtggtactctgttattacggtaactttgtacgccagttttatctcccttcccccatgtaacttagaagtttttcacaaagaccaatagccggtaatcagccagattactgaaggtcaagcacttctgtttccccggtcaatgttgatatgctccaacagggcaaaaacaactgcgatcgttatccgcaaagcgcctacgcaaagcttagtagcatctttgaaatcgtttggctggtcgatccgccatttcccctggtagacctggcagatgaggctagaaataccccactggcgacagtgttctagcctgcgtggctgcctgcacaccctatgggtgtgaagccaaacaatggacaaggtgtgaagagccccgtgtgctcgctttgagtcctccggcccctgaatgtggctaaccttaaccctgcagctagagcacgtaacccaacgtgtatctagtcgtaatgagcaattgcgggatgggaccaactactttgggtgtccgtgtttcactttttcctttatatttgcttatggtgacaatatatacaatatatatattg

SEQ ID NO: 121 - DNA, 19 bp, synthetic construct
  misc_feature 1..19: note = Synthetic Oligonucleotide
  source 1..19: mol_type = other DNA
yrgrcytggcagatgrggc

SEQ ID NO: 122 - DNA, 19 bp, synthetic construct
  misc_feature 1..19: note = Synthetic Oligonucleotide
  source 1..19: mol_type = other DNA
taracctggcagatgrggc

SEQ ID NO: 123 - DNA, 19 bp, synthetic construct
  misc_feature 1..19: note = Synthetic Oligonucleotide
  source 1..19: mol_type = other DNA
tagacctggcagatggggc

SEQ ID NO: 124 - DNA, 19 bp, synthetic construct
  misc_feature 1..19: note = Synthetic Oligonucleotide
  source 1..19: mol_type = other DNA
tagacctggcagatgrggc

SEQ ID NO: 125 - DNA, 19 bp, synthetic construct
  misc_feature 1..19: note = Synthetic Oligonucleotide
  source 1..19: mol_type = other DNA
taracctggcagatggggc

SEQ ID NO: 126 - DNA, 19 bp, synthetic construct
  misc_feature 1..19: note = Synthetic Oligonucleotide
  source 1..19: mol_type = other DNA
taracctggtagatgrggc

SEQ ID NO: 127 - DNA, 17 bp, synthetic construct
  misc_feature 1..17: note = Synthetic Oligonucleotide
  source 1..17: mol_type = other DNA
taracctggcagatgrg

SEQ ID NO: 128 - DNA, 18 bp, synthetic construct
  misc_feature 1..18: note = Synthetic Oligonucleotide
  source 1..18: mol_type = other DNA
taracctggcagatgrgg

SEQ ID NO: 129 - DNA, 19 bp, synthetic construct
  misc_feature 1..19: note = Synthetic Oligonucleotide
  source 1..19: mol_type = other DNA
caracctggcagatgrggc

SEQ ID NO: 130 - DNA, 15 bp, synthetic construct
  misc_feature 1..15: note = Synthetic Oligonucleotide
  source 1..15: mol_type = other DNA
cctgccagatgrggc

SEQ ID NO: 131 - DNA, 19 bp, synthetic construct
  misc_feature 1..19: note = Synthetic Oligonucleotide
  source 1..19: mol_type = other DNA
wgcctgcgyggckgccwrc

SEQ ID NO: 132 - DNA, 17 bp, synthetic construct
  misc_feature 1..17: note = Synthetic Oligonucleotide
  source 1..17: mol_type = other DNA
ccygcgcggctgcctrc

SEQ ID NO: 133 - DNA, 17 bp, synthetic construct
  misc_feature 1..17: note = Synthetic Oligonucleotide
  source 1..17: mol_type = other DNA
ccygcgtggctgcctrc

SEQ ID NO: 134 - DNA, 17 bp, synthetic construct
  misc_feature 1..17: note = Synthetic Oligonucleotide
  source 1..17: mol_type = other DNA
ccygcgtggctgcctgc

SEQ ID NO: 135 - DNA, 19 bp, synthetic construct
  misc_feature 1..19: note = Synthetic Oligonucleotide
  source 1..19: mol_type = other DNA
wgccygcgtggctgcctgc

SEQ ID NO: 136 - DNA, 19 bp, synthetic construct
  misc_feature 1..19: note = Synthetic Oligonucleotide
  source 1..19: mol_type = other DNA
agccygcgtggctgcctgc

SEQ ID NO: 137 - DNA, 27 bp, synthetic construct
  misc_feature 1..27: note = Synthetic Oligonucleotide
  source 1..27: mol_type = other DNA
grttagccgcattcrggrgccggagga

SEQ ID NO: 138 - DNA, 46 bp, synthetic construct
  misc_feature 1..46: note = Synthetic Oligonucleotide
  source 1..46: mol_type = other DNA
tacatgcacatckcsggvcaggaygcytcggagtacctgagccccg

SEQ ID NO: 139 - DNA, 22 bp, synthetic construct
  misc_feature 1..22: note = Synthetic Oligonucleotide
  source 1..22: mol_type = other DNA
acgcctcggagtacctgagccc

SEQ ID NO: 140 - DNA, 24 bp, synthetic construct
  misc_feature 1..24: note = Synthetic Oligonucleotide
  source 1..24: mol_type = other DNA
cggggctcaggtactccgaggcgt

SEQ ID NO: 141 - DNA, 22 bp, synthetic construct
  misc_feature 1..22: note = Synthetic Oligonucleotide
  source 1..22: mol_type = other DNA
gtkgcrcgggcraaytgcacca

SEQ ID NO: 142 - DNA, 18 bp, synthetic construct
  misc_feature 1..18: note = Synthetic Oligonucleotide
  source 1..18: mol_type = other DNA
gtkgcrcgggcgaactgc

SEQ ID NO: 143 - DNA, 17 bp, synthetic construct
  misc_feature 1..17: note = Synthetic Oligonucleotide
  source 1..17: mol_type = other DNA
gtggcgcgggcaaactg

SEQ ID NO: 144 - DNA, 18 bp, synthetic construct
  misc_feature 1..18: note = Synthetic Oligonucleotide
  source 1..18: mol_type = other DNA
gtkgcrcgggcraactgc

SEQ ID NO: 145 - DNA, 18 bp, synthetic construct
  misc_feature 1..18: note = Synthetic Oligonucleotide
  source 1..18: mol_type = other DNA
gtggcrcgggcraactgc

SEQ ID NO: 146 - DNA, 18 bp, synthetic construct
  misc_feature 1..18: note = Synthetic Oligonucleotide
  source 1..18: mol_type = other DNA
gtkgcgcgggcraactgc

SEQ ID NO: 147 - DNA, 18 bp, synthetic construct
  misc_feature 1..18: note = Synthetic Oligonucleotide
  source 1..18: mol_type = other DNA
gtggcgcgggcraactgc

SEQ ID NO: 148 - DNA, 18 bp, synthetic construct
  misc_feature 1..18: note = Synthetic Oligonucleotide
  source 1..18: mol_type = other DNA
gtggcrcgggcgaactgc

SEQ ID NO: 149 - DNA, 18 bp, synthetic construct
  misc_feature 1..18: note = Synthetic Oligonucleotide
  source 1..18: mol_type = other DNA
gtkgcgcgggcgaactgc

SEQ ID NO: 150 - DNA, 13293 bp, Human Metapneumovirus
  source 1..13293: mol_type = unassigned DNA
acgcgaaaaaaacgcgtataaattaaattccaaacaaaacgggacaaataaaaatgtctcttcaagggattcacctaagtgatctatcatataaacatgctatattaaaagagtctcaatacacaataaaaagagatgtaggcaccacaactgcagtgacaccttcatcattacaacaagaaataacacttttgtgtggggaaatactttacactaaacacactgattacaaatatgctgctgagataggaatacaatatatttgcacagctctaggatcagaaagagtacaacagattttgagaaactcaggtagtgaagttcaggtggttctaaccaaaacatactccttagggaaaggcaaaaacagtaaaggggaagagctgcagatgttagatatacatggagtggaaaagagttggatagaagaaatagacaaagaggcaagaaagacaatggtaactttgcttaaggaatcatcaggtaacatcccacaaaaccagagaccttcagcaccagacacaccaataattttattatgtgtaggtgccctaatattcactaaactagcatcaacaatagaagttggattagagactacagttagaagagctaatagagtgctaagtgatgcactcaaaagatacccaaggatagatataccaaagattgctagatctttttatgaactatttgaacaaaaagtgtactacagaagtttattcattgagtacggaaaagctttaggctcatcttcaacaggaagcaaagcagaaagtttgtttgtaaatatatttatgcaagcttatggagctggccaaacactgctaaggtggggtgtcattgccagatcatccaacaacataatgctagggcatgtatctgtgcaatctgaattgaagcaagttacagaggtttatgacttggtgagagaaatgggtcctgaatctgggcttttacatctaagacaaagtccaaaggcagggctgttatcattggccaattgccccaattttgctagtgttgttcttggcaatgcttcaggtctaggcataatcggaatgtacagagggagagtaccaaacacagagctattttctgcagcagaaagttatgccagaagcttaaaagaaagcaataaaatcaacttctcttcgttagggcttacagatgaagaaaaagaagctgcagaacacttcttaaacatgagtggtgacaatcaagatgattatgagtaattaaaaaactgggacaagtcaaaatgtcattccctgaaggaaaggatattctgttcatgggtaatgaagcagcaaaaatagccgaagctttccagaaatcactgaaaaaatcaggtcacaagagaactcaatctattgtaggggaaaaagttaacactatatcagaaactctagaactacctaccatcagcaaacctgcacgatcatctacactgctggaaccaaaattggcatgggcagacaacagcggaatcaccaaaatcacagaaaaaccagcaaccaaaacaacagatcctgttgaagaagaggaattcaatgaaaagaaagtgttaccttccagtgatgggaagactcctgcagagaaaaaatcaaagttttcaaccagtgtaaaaaagaaagtttcctttacatcaaatgaaccagggaaatacaccaaactagagaaagatgccctagatttgctctcagacaatgaggaagaagacgcagaatcctcaatcctaacttttgaggagaaagatacatcatcactaagcattgaagctagactagaatctatagaagagaagttgagcatgatattaggactgcttcgtacacttaacattgcaacagcaggaccaacagctgcacgagatggaattagggatgcaatgattggtataagagaagagctaatagcagagataattaaggaagccaagggaaaagcagctgaaatgatggaagaagagatgaatcaaagatcaaaaataggaaatggcagtgtaaaactaaccgagaaggcaaaagagctcaacaaaattgttgaagacgagagcacaagcggtgaatcagaagaagaagaagaaccaaaagaaactcaggataacaatcaaggagaagatatttatcagttaatcatgtagtttaataaaaataaacaatgggacaagtcaagatggagtcctatctagtagacacttatcaaggcattccatatacagctgctgttcaagttgacctggtagaaaaagatttactgccagcaagtttgacaatatggtttcctttatttcaggccaacacaccaccagcagttctgcttgatcagctaaaaaccttgacaataacaactctgtatgctgcatcacagaatggtccaatactcaaggtaaatgcatctgcccaaggtgctgccatgtctgtacttcccaaaaaattcgaggtaaatgcaactgtagcacttgatgaatacagtaaacttgattttgacaagctgacggtctgcgatgttaaaacagtttatttgacaactatgaaaccgtacgggatggtgtcaaaatttgtgagttcagccaaatcagttggcaaaaagacacatgatctaattgcactatgtgacttcatggacctagagaaaaatatacctgtgacaataccagcattcataaagtcagtttcaatcaaagagagtgaatcagccactgttgaagctgcaataagcagcgaagccgaccaagccttgacacaagccaagattgcgccctatgcaggactaattatgatcatgaccatgaacaatccaaaaggtatattcaagaaactaggggctggaacacaagtgatagtagagctgggggcatatgttcaggctgagagcatcagtaggatctgcaagagctggagtcaccaaggaacaagatacgtactaaaatccagataaaaataactgtcttaatcaataattgcttatataactctagagattaataagcttattattatagttatataaaaataaattagaattagaagggcatcaatagaaagcgggacaaataaaaatgtcttggaaagtgatgatcatcatttcgttactcataacaccccagcacgggctaaaggagagttatttggaagaatcatgtagtactataactgagggatacctcagtgttttaagaacaggctggtacactaatgtcttcacattagaagttggtgatgttgaaaatcttacatgtactgatggacctagcttaatcaaaacagaacttgatctaacaaaaagtgctttaagggaactcaaaacagtctctgctgatcagttggcgagagaggagcaaattgaaaatcccagacaatcaagatttgtcttaggtgcgatagctctcggagttgctacagcagcagcagtcacagcaggcattgcaatagccaaaaccataaggcttgagagtgaggtgaatgcaattaaaggtgctctcaaacaaactaatgaagcagtatccacattagggaatggtgtgcgggtcctagccactgcagtgagagagctaaaagaatttgtgagcaaaaacctgactagtgcaatcaacaggaacaaatgtgacattgctgatctgaagatggctgtcagcttcagtcaattcaacagaagatttctaaatgttgtgcggcagttttcagacaatgcagggataacaccagcaatatcattggacctgatgactgatgctgagttggccagagctgtatcatacatgccaacatctgcagggcagataaaactgatgttggagaaccgcgcaatggtaaggagaaaaggatttggaatcctgataggggtctacggaagctctgtgatttacatggttcaattgccgatctttggtgtcatagatacaccttgttggatcatcaaggcagctccctcttgctcagaaaaaaacgggaattatgcttgcctcctaagagaggatcaagggtggtattgtaaaaatgcaggatctactgtttactacccaaatgaaaaagactgcgaaacaagaggtgatcatgttttttgtgacacagcagcagggatcaatgttgctgagcaatcaagagaatgcaacatcaacatatctactaccaactacccatgcaaagtcagcacaggaagacaccctataagcatggttgcactatcacctctcggtgctttggtggcttgctataaaggggtaagctgctcgattggcagcaattgggttggaatcatcaaacaattacccaaaggctgctcatacataaccaaccaggatgcagacactgtaacaattgacaataccgtgtatcaactaagcaaagttgaaggtgaacagcatgtaataaaagggagaccagtttcaagcagttttgatccaatcaagtttcctgaggatcagttcaatgttgcgcttgatcaagtcttcgaaagcattgagaacagtcaggcactagtggaccagtcaaacaaaattctaaacagtgcagaaaaaggaaacactggtttcattatcgtagtaattttggttgctgttcttggtctaaccatgatttcagtgagcatcatcatcataatcaagaaaacaaggaagcccacaggagcacctccagagctgaatggtgtcaccaacggcggtttcataccacatagttagttaattaaaaaatgggacaaatcatcatgtctcgtaaggctccatgcaaatatgaagtgcggggcaaatgcaacagagggagtgattgcaaattcaatcacaattactggagttggcctgatagatatttattgttaagatcaaattatctcttaaatcagcttttaagaaacacagataaggctgatggtttgtcaataatatcaggagcaggtagagaagatagaactcaagactttgttcttggttctactaatgtggttcaagggtacattgatgacaaccaaggaataaccaaggctgcagcttgctatagtctacacaacataatcaagcaactacaagaaacagaagtaagacaggctagagacaacaagctttctgatagcaaacatgtggcgctccacaacttgatattatcctatatggagatgagcaaaactcctgcatctctaatcaacaacctaaagaaactaccaagggaaaaactgaagaaattagcaagattaataattgatttatcagcaggaactgacaatgactcttcatatgccttgcaagacagtgaaagcactaatcaagtgcagtaaacatggtcccaaattcattaccatagaggcagatgatatgatatggactcacaaagaattaaaagaaacactgtctgatgggatagtaaaatcacacaccaatatttatagttgttacttagaaaatatagaaataatatatgttaaaacttacttaagttagtaaaaaataaaaatagaatgggataaatgacaatgaaaacattagatgtcataaaaagtgatggatcctcagaaacgtgtaatcaactcaaaaaaataataaaaaaacactcaggtaaagtgcttattgcactaaaactgatattggccttactgacatttttcacagcaacaatcactgtcaactatataaaagtagaaaacaatttgcaggcatgtcaaccaaaaaatgaatcagacaaaaaggtcacaaagccaaataccacatcaacaacaatcagacccacacccgatccaactgtagtacatcatttgaaaaggctgattcagagacacaccaactctgtcacaaaagacagcgatacttgttggagaatacacaagaatcaacgtacaaatataaaaatatacaagttcttatgctctgggttcacaaattcaaaaggtacagattgtgaggaaccaacagccctatgcgacaaaaagttaaaaaccatagtagaaaaacatagaaaagcagaatgtcactgtctacatacaaccgagtgggggtgccttcatccctaaaataacacggctttcaacattaaaatcagaacaacctccacccaggtctatcaatacagtggtttagccatttaaaaaccgaatattatctaggctgcacgacactttgcaataatatgcaatagtcaatagttaaaccactgctgcaaactcatccataatataatcactgagtaatacaaaacaagaaaatgggacaagtggctatggaagtaagagtggagaacattcgagcgatagacatgttcaaagcaaagataaaaaaccgtataagaagcagcaggtgctatagaaatgctacactgatccttattggactaacagcgttaagcatggcacttaatattttcctgatcatcgatcatgcaacattaagaaacatgatcaaaacagaaaactgtgctaacatgccgtcggcagaaccaagcaaaaagaccccaatgacctccacagcaggcccaaacaccaaacccaatccacagcaagcaacacagtggaccacagagaactcaacatccccagtagcaaccccagagggccatccatacacagggacaactcaaacatcagacacaacagctccccagcaaaccacagacaaacacacagcaccgctaaaatcaaccaatgaacagatcacccagacaaccacagagaaaaagacaatcagagcaacaacccaaaaaagggaaaaaggaaaagaaaacacaaaccaaaccacaagcacagctgcaacccaaacaaccaacaccaccaaccaaatcagaaatgcaagtgagacaatcacaacatccgacagacccagaactgacaccacaacccaaagcagcgaacagacaacccgggcaacagacccaagctccccaccacaccatgcatagagaggtgcaaaactcaaatgagcacaacacacaaacatcccatccaagtagttaacaaaaaaccacaaaataaccttgaaaaccaaaaaaccaaaacataaacccagacccagaaaaacatagacaccatatggaaggttctagcatatgcaccaatgagatggcatctgttcatgtatcaatagcaccaccatcattcaaggaataagaagaggcgaaaatttaagggataaatgacaatggatcccttttgtgaatctactgttaatgtttatctccctgattcatatctcaaaggagtaatatcttttagtgaaaccaatgcaattggatcatgtcttttgaaaagaccctatctaaaaaatgacaacactgccaaagttgctgtagaaaaccctgttgttgaacatgtgaggcttagaaatgcagtcatgaccaaaatgaagatatcagattataaagtggttgaaccagttaatatgcagcatgaaataatgaaaaatatacatagttgtgagcttacattattaaaacaattcttaacgagaagcaaaaacattagctctctaaaattaaatatgatatgtgattggttacagttaaaatccacttcagataacacatcaattctcaattttatagatgtggagttcatacccgtttgggtaagcaattggttcagtaactggtataatctcaataaattaatcttagagtttagaagagaagaagtaataagaactggttcaattttatgtagatcactaggcaagttagtttttattgtatcatcttatggatgtgtagtaaaaagcaacaaaagtaaaagagtgagctttttcacctataaccaactgttaacatggaaagatgtgatgttaagtagattcaatgcaaacttttgtatatgggtaagtaacaacctgaacaaaaatcaagaaggactaggacttagaagcaatctgcaaggtatgttaaccaataaattatatgaaactgttgattacatgctaagcctatgctgcaatgaaggattctctctggtgaaagagtttgaaggatttattatgagtgaaattctaaaaattactgagcatgctcagttcagtactaggtttaggaatactttattgaatgggttaactgaacaattatcagtgttgaaagctaagaacagatctagagttcttggaactatattagaaaacaacaattaccctatgtacgaagtagtacttaaattattaggggacaccttgaaaagcataaagttattaattaacaagaatttagaaaatgctgcagaattatattatatattcagaatttttggacaccctatggtagatgagagggaagcaatggatgctgttaaattaaacaatgagattacaaaaattcttaaattagagagtttaacagaactaagaggagcatttatactaagaattataaaagggtttgtagacaataataaaagatggcctaaaattaagaatttaaaagtgctcagcaaaagatgggctatgtatttcaaagctaaaagttaccctagccaacttgagctaagtgtacaagattttttagaacttgctgcagtacaatttgagcaggaattctctgtacctgaaaaaaccaaccttgagatggtattaaatgataaagcaatatcacctccaaaaaagctaatatggtctgtatatccaaaaaactacctgcctgaaactataaaaaatcaatatttagaagaggctttcaatgcaagtgacagccaaagaacaaggagagtcttagaattttacttaaaagattgtaaatttgatcaaaaagaacttaaacgttatgtaattaaacaagagtatctgaatgacaaagaccacattgtctcgttaactgggaaggaaagagaattaagtgtaggtaggatgtttgcaatgcaaccaggaaaacaaagacagatacagatattagctgagaaacttctagctgataatattgtaccttttttcccagaaactttaacaaagtatggtgacttagatctccaaagaattatggaaataaaatcagaactttcttccattaaaactagaaagaatgatagctacaacaattatattgcaagggcctctatagtaacagacttaagtaagttcaatcaggcctttagatatgaaaccacagctatatgtgcagatgtagctgatgagttacatgggacacaaagcttattctgttggttacatcttattgttcccatgactacaatgatatgtgcatacagacatgcaccaccagaaacaaaaggggaatatgatatagacaaaatacaagagcaaagcggattatacagatatcatatgggagggattgaagggtggtgccagaagttatggacaatggaagcaatatccttgttagatgtagtatctgtgaagactcgctgtcagatgacctctctattaaacggagacaatcagtcaatagatgttagtaaaccagtaaaattgtctgaaggtatagatgaagtaaaagcagactatagcttagcaattagaatgcttaaagaaataagagatgcttataaaaacattggtcataaactcaaagaaggtgaaacatatatatcaagggatctccaatttataagtaaggtgattcaatctgaaggagtcatgcatcctacccctataaaaaagatattaagagtaggtccttggataaatacaatactagatgatattaaaaccagtgcagaatcaataggaagtctatgtcaagaactagaattcagaggggagagtatactagttagcttgatattaaggaatttctggctgtataacttgtacatgtatgagtcaaaacagcacccattagctgggaagcaactgttcaagcaattgaacaaaacattaacatctgtgcagagattttttgaactgaagaaagaaaatgatgtggttgacctatggatgaatataccaatgcagtttggagggggagatccagtagttttttacagatctttttacagaaggactcccgatttcctaactgaagcaatcagccatgtggatttactgttaaaagtgtcaaacaatatcaaagatgagactaagatacgatttttcaaagccttattatctatagaaaagaatgaacgtgctacattaacaacactaatgagagaccctcaggcagtaggatcagaacgacaagctaaggtaacaagtgatataaatagaacagcagttaccagcatactgagtctatctccgaatcagctcttctgtgatagtgctatacattatagtagaaatgaggaagaagttgggatcattgcagacaacataacacctgtctatcctcatgggctgagagtgctctatgaatcactaccttttcataaggctgaaaaggttgtcaatatgatatcaggcacaaagtctataactaatctattacagagaacatctgctatcaatggtgaagatattgatagagcagtgtctatgatgttagagaacttagggttgttatctagaatattgtcagtaataattaatagtatagaaataccaatcaagtccaatggcagattgatatgctgtcaaatttccaagaccttgagagaaaaatcatggaacaatatggaaatagtaggagtgacatctcctagtattgtgacatgtatggatgttgtgtatgcaactagttctcatttaaaaggaataattattgaaaaattcagtactgacaagaccacaagaggtcagaggggaccaaaaagcccctgggtaggatcaagcactcaagagaaaaaattggttcctgtttataatagacaaattctttcaaaacaacaaaaagagcaactggaagcaatagggaaaatgaggtgggtgtacaaaggaactccagggctaagaagattgctcaacaagatttgcataggaagcttaggtattagctataaatgtgtgaaacctttattaccaagattcatgagtgtaaacttcttacataggttatctgttagtagtagacccatggaattcccagcttctgttccagcttacaggacaacaaattaccattttgacactagtccaatcaaccaagcattaagtgagaggttcgggaacgaagacattaatttagtgttccaaaatgcaatcagctgcggaattagtataatgagtgttgtagaacagttaactggtagaagcccaaaacaattagtcctaatccctcaattagaagagatagatattatgcctcctcctgtatttcaaggaaaattcaattataaactagttgataagataacctccgatcaacacatcttcagtcctgacaaaatagacatattaacactagggaagatgcttatgcctaccataaaaggtcaaaaaactgatcagttcttaaataagagagaaaactattttcatggaaataatttaattgaatctttatctgcagcacttgcatgccactggtgtgggatattaacagaacagtgcatagaaaacaatatctttaggaaagattggggtgatgggttcatctcagatcatgccttcatggatttcaaggtatttctatgtgtatttaaaaccaaacttttatgtagttggggatctcaaggaaagaatgtaaaagatgaagatataatagatgaatccattgacaaattattaagaattgacaacaccttttggagaatgttcagcaaagtcatgtttgaatcaaaagtcaaaaaaagaataatgttatatgatgtgaaattcctatcattagtaggttatataggatttaaaaactggtttatagaacagttaagagtggtagaattgcatgaggtaccttggattgtcaatgctgaaggagagttagttgaaattaaatcaatcaaaatttatctgcagttaatagaacaaagtctatctttgagaataactgtattgaattatacagacatggcacatgctcttacacgattaattaggaaaaaattgatgtgtgataatgcactctttaatccaagttcatcaccaatgtttaatctaactcaggttattgatcccacaacacaactagactattttcctaggataatatttgagaggttaaaaagttatgataccagttcagactacaacaaagggaagttaacaaggaattacatgacattattaccatggcaacacgtaaacaggtacaattttgtctttagttctacaggttgtaaagtcagtttgaagacatgcatcgggaaattgataaaggatttaaatcctaaagttctttactttattggagaaggagcaggtaactggatggcaagaacagcatgtgaatatcctgatataaaatttgtatataggagtttaaaggatgaccttgatcaccattacccattagaatatcaaagggtaataggtgatctaaatagggtgatagatagtggtgaaggattatcaatggaaaccacagatgcaactcaaaaaactcattgggacttgatacacagaataagtaaagatgctttattgataacattgtgtgatgcagaattcaaaaacagagatgatttctttaagatggtaatcctttggagaaaacatgtattatcttgtagaatctgtacagcttatggaacagatctttacttatttgcaaagtatcatgcggtggactgcaatataaaattaccattttttgtaagatctgtagctacttttattatgcaaggaagcaaattatcagggtcagaatgttacatacttttaacattaggtcatcacaataatctaccctgtcatggagaaatacaaaattccaaaatgagaatagcagtgtgtaatgatttctatgcctcaaagaaactggacaacaaatcaattgaagcaaactgcaaatctcttctatcaggattgagaatacctataaacaaaaaggagttaaatagacaaaagaaattgttaacactacaaagtaaccattcttctatagcaacagttggcggcagtaagattatagaatccaaatggttaaagaataaagcaagtacaataattgattggttagagcatattttgaattctccaaaaggtgaattaaactatgatttctttgaagcattagagaacacataccccaatatgatcaagcttatagataatttgggaaatgcagaaataaagaaactaatcaaggtcactgggtatatgcttgtgagtaagaagtaataataatgataatgattaaccataatctcacacaactgagaaaataatcgtctaacagtttagttgatcattagttatttaaaattataaaatagtaactaactgataaaaaatcagaaattgaaattgaatgtatacggtttttttgccgt

SEQ ID NO: 151 - DNA, 28 bp, synthetic construct
  misc_feature 1..28: note = Synthetic Oligonucleotide
  source 1..28: mol_type = other DNA
cssccaattttgctagtgttgttcttgg

SEQ ID NO: 152 - DNA, 28 bp, synthetic construct
  misc_feature 1..28: note = Synthetic Oligonucleotide
  source 1..28: mol_type = other DNA
cggccaattttgctagtgttgttcttgg

SEQ ID NO: 153 - DNA, 24 bp, synthetic construct
  misc_feature 1..24: note = Synthetic Oligonucleotide
  source 1..24: mol_type = other DNA
caattttgctagtgttgttcttgg

SEQ ID NO: 154 - DNA, 25 bp, synthetic construct
  misc_feature 1..25: note = Synthetic Oligonucleotide
  source 1..25: mol_type = other DNA
ccaattttgctagtgttgttcttgg

SEQ ID NO: 155 - DNA, 36 bp, synthetic construct
  misc_feature 1..36: note = Synthetic Oligonucleotide
  source 1..36: mol_type = other DNA
tgcttcaggtytaggyataatcggaatgtwcagagg

SEQ ID NO: 156 - DNA, 36 bp, synthetic construct
  misc_feature 1..36: note = Synthetic Oligonucleotide
  source 1..36: mol_type = other DNA
tgcttcaggtttaggcataatcggaatgttcagagg

SEQ ID NO: 157 - DNA, 29 bp, synthetic construct
  misc_feature 1..29: note = Synthetic Oligonucleotide
  source 1..29: mol_type = other DNA
tgcttcaggtctaggtataatcggaatgt

SEQ ID NO: 158 - DNA, 23 bp, synthetic construct
  misc_feature 1..23: note = Synthetic Oligonucleotide
  source 1..23: mol_type = other DNA
gcagaaaatagctctgtgtttgg

SEQ ID NO: 159 - DNA, 1045 bp, Human Metapneumovirus
  source 1..1045: mol_type = unassigned DNA
cacaataaagagagatgtgggcacaacaacagcagtaacaccctcatcattgcaacaagaaataacactgttgtgtggagaaattctatatgctaagcatactgattacaaatatgctgcagaaataggaatacaatatattagcacagctctagggtcagagagagtacagcagattctaagaaactcaggcagtgaagtccaagcggttttaaccagaacgtactctttggggaaagttaaaaacaataaaggagaagatttacagatgttagacatacatggagtagaaaaaagctgggtggaagagatagacaaagaagcaagaaaaacaatggcaactttacttaaagaatcatcaggcaatattccacaaaatcagaggccttcagcaccagacacacctataatcttattatgtgtaggtgccttaatatttaccaaactagcatcaactatagaagtgggattagagaccacagtcagaagagctaaccgtgtactaagtgatgcactcaaaagataccctagaatggacataccaaaaattgctagatccttctatgacttatttgaacaaaaagtgtatcacagaagtttgttcattgagtatggcaaagcattaggctcatcctctacaggcagcaaagcagaaagtttattcgtcaacatattcatgcaagcttatggtgctggtcaaacaatgctgaggtggggggttatcgccaggtcatctaacaatataatgttaggacatgtatctgtacaagccgagctgaaacaggtcacagaagtctatgacctagtgcgggaaatgggccctgaatctgggctcctacatttaaggcaaagcccaaaagctggactgttatcccttgcaaattgtcccaactttgcaagtgttgttctcggcaatgcctcaggcttaggcataataggtatgtatcgagggagagtgccaaacacagaactattttcagcagcagaaagctatgccaagagtttgaaagaaagtaataaaatcaacttttcttcattaggactc

SEQ ID NO: 160 - DNA, 21 bp, synthetic construct
  misc_feature 1..21: note = Synthetic Oligonucleotide
  source 1..21: mol_type = other DNA
ctttgcaagtgttgttctcgg

SEQ ID NO: 161 - DNA, 37 bp, synthetic construct
  misc_feature 1..37: note = Synthetic Oligonucleotide
  source 1..37: mol_type = other DNA
tgcctcaggcytaggcataatmggyatgtatcghggg

SEQ ID NO: 162 - DNA, 29 bp, synthetic construct
  misc_feature 1..29: note = Synthetic Oligonucleotide
  source 1..29: mol_type = other DNA
tcaggcttaggcataataggtatgtatcg

SEQ ID NO: 163 - DNA, 33 bp, synthetic construct
  misc_feature 1..33: note = Synthetic Oligonucleotide
  source 1..33: mol_type = other DNA
cctcaggcttaggcataataggtatgtatcgag

SEQ ID NO: 164 - DNA, 31 bp, synthetic construct
  misc_feature 1..31: note = Synthetic Oligonucleotide
  source 1..31: mol_type = other DNA
cctcaggcttaggcataataggtatgtatcg

SEQ ID NO: 165 - DNA, 33 bp, synthetic construct
  misc_feature 1..33: note = Synthetic Oligonucleotide
  source 1..33: mol_type = other DNA
cctcaggcttaggcataataggtatgtatcgcg

SEQ ID NO: 166 - DNA, 33 bp, synthetic construct
  misc_feature 1..33: note = Synthetic Oligonucleotide
  source 1..33: mol_type = other DNA
  modified_base 32: mod_base = OTHER; note = uracil
cctcaggcttaggcataataggtatgtatcgtg

SEQ ID NO: 167 - DNA, 37 bp, synthetic construct
  misc_feature 1..37: note = Synthetic Oligonucleotide
  source 1..37: mol_type = other DNA
  modified_base 34: mod_base = OTHER; note = uracil
tgcctcaggcctaggcataatcggcatgtatcgtggg

SEQ ID NO: 168 - DNA, 37 bp, synthetic construct; identical to SEQ ID NO: 167
  misc_feature 1..37: note = Synthetic Oligonucleotide
  source 1..37: mol_type = other DNA

SEQ ID NO: 169 - DNA, 32 bp, synthetic construct
  misc_feature 1..32: note = Synthetic Oligonucleotide
  source 1..32: mol_type = other DNA
ctcaggcttaggcataataggtatgtatcgcg

SEQ ID NO: 170 - DNA, 34 bp, synthetic construct
  misc_feature 1..34: note = Synthetic Oligonucleotide
  source 1..34: mol_type = other DNA
tgcctcaggcttaggcataataggtatgtatcgc

SEQ ID NO: 171 - DNA, 35 bp, synthetic construct
  misc_feature 1..35: note = Synthetic Oligonucleotide
  source 1..35: mol_type = other DNA
tgcctcaggcttaggcataataggtatgtatcgcg

SEQ ID NO: 172 - DNA, 36 bp, synthetic construct
  misc_feature 1..36: note = Synthetic Oligonucleotide
  source 1..36: mol_type = other DNA
tgcctcaggcttaggcataataggtatgtatcgcgg

SEQ ID NO: 173 - DNA, 37 bp, synthetic construct
  misc_feature 1..37: note = Synthetic Oligonucleotide
  source 1..37: mol_type = other DNA
  modified_base 34: mod_base = OTHER; note = uracil
tgcctcaggcttaggcataataggtatgtatcgtggg

SEQ ID NO: 174 - DNA, 37 bp, synthetic construct
  misc_feature 1..37: note = Synthetic Oligonucleotide
  source 1..37: mol_type = other DNA
tgcctcaggcttaggcataataggtatgtatcgaggg

SEQ ID NO: 175 - DNA, 37 bp, synthetic construct
  misc_feature 1..37: note = Synthetic Oligonucleotide
  source 1..37: mol_type = other DNA
tgcctcaggcttaggcataatcggtatgtatcgcggg

SEQ ID NO: 176 - DNA, 37 bp, synthetic construct
  misc_feature 1..37: note = Synthetic Oligonucleotide
  source 1..37: mol_type = other DNA
tgcctcaggcttaggcataataggtatgtatcgcggg

SEQ ID NO: 177 - DNA, 28 bp, synthetic construct
  misc_feature 1..28: note = Synthetic Oligonucleotide
  source 1..28: mol_type = other DNA
ctgctgcwgaaaatagytctgtgtttgg

SEQ ID NO: 178 - DNA, 24 bp, synthetic construct
  misc_feature 1..24: note = Synthetic Oligonucleotide
  source 1..24: mol_type = other DNA
tgctgaaaatagttctgtgtttgg